European Patent Specification EP 3 250 191 B1, published January 17, 2024. Title: TABLETS COMPRISING GLP-1 AGONIST AND ENTERIC COATING. Applicant: Novo Nordisk A/S. The sequence listing filed with the application follows.

SEQUENCE LISTING (10 sequences)

SEQ ID NO: 1 - protein, 31 aa, Homo sapiens
HAEGTFTSDVSSYLEGQAAKEFIAWLVKGRG

SEQ ID NO: 2 - protein, 39 aa, Heloderma suspectum
HSDGTFTSDLSKQMEEEAVRLFIEWLKNGGPSSGAPPPS

SEQ ID NO: 3 - protein, 39 aa, Heloderma suspectum
HGEGTFTSDLSKQMEEEAVRLFIEWLKNGGPSSGAPPPS

SEQ ID NO: 4 - protein, 33 aa, ARTIFICIAL
  Based on human GLP-1
  SITE (1)..(1): This residue is L-His, imidazopropionyl, alpha-hydroxy-histidine, D-His, desamino-His, 2-amino-His, beta-hydroxy-His, homo-His, N-alpha-acetyl-His, N-alpha-formyl-His, alpha-fluoromethyl-His, alpha-methyl-His, 3-pyridyl-Ala, 2-pyridyl-Ala, or 4-pyridyl-Ala
  SITE (2)..(2): This residue is Ala, Gly, Val, Leu, Ile, Thr, Ser, Lys, Aib, (1-aminocyclopropyl) carboxylic acid, (1-aminocyclobutyl) carboxylic acid (CA), (1-aminocyclopentyl) CA, (1-aminocyclohexyl) CA, (1-aminocycloheptyl) CA, or
  SITE (6)..(6): This residue is Lys or Phe
  SITE (10)..(10): This residue is Val or Leu
  SITE (12)..(12): This residue is Ser, Arg, Asn, Gln, or Glu
  SITE (13)..(13): This residue is Tyr or Gln
  SITE (14)..(14): This residue is Leu, Lys, or Met
  SITE (16)..(16): This residue is Gly, Glu, Lys, or Aib
  SITE (17)..(17): This residue is Gln, Glu, or Arg
  SITE (18)..(18): This residue is Ala or Lys
  SITE (19)..(19): This residue is Ala or Val
  SITE (20)..(20): This residue is Val, His, Lys or Arg
  SITE (24)..(24): This residue is Ala, Glu, or Arg
  SITE (25)..(25): This residue is Trp or His
  SITE (28)..(28): This residue is Glu, Asn, Gly, Gln, or Arg
  SITE (29)..(29): This residue is Gly, Aib, or absent
  SITE (30)..(30): This residue is Arg, Gly, Lys, or absent
  SITE (31)..(31): This residue is Gly, Ala, Glu, Pro, Lys, Arg, or absent
  SITE (32)..(32): This residue is Ser, Gly, Ala, Glu, Gln, Pro, Arg, or absent
  SITE (33)..(33): This residue is Gly or absent
XXEGTXTSDXSXXXEXXXXXKFIXXLVXXXXXX

SEQ ID NO: 5 - protein, 31 aa, ARTIFICIAL
  Based on human GLP-1
  SITE (2)..(2): This amino acid residue is Aib
  SITE (20)..(20): This amino acid residue is covalently attached to a substituent
  SITE (31)..(31): This amino acid residue is covalently attached to a substituent
HXEGTFTSDVSSYLEGQAAKEFIAWLVRGRK

SEQ ID NO: 6 - protein, 33 aa, ARTIFICIAL
  Based on human GLP-1
  SITE (2)..(2): This amino acid residue is Aib
  SITE (21)..(21): This amino acid residue is covalently attached to a substituent
  SITE (30)..(30): This amino acid residue is covalently attached to a substituent
HXEGTFTSDVSSYLEEQAARKFIGWLVRGKGEG

SEQ ID NO: 7 - protein, 31 aa, ARTIFICIAL
  Based on human GLP-1
  SITE (1)..(1): This residue (Xaa7) is L-His, (S)-2-Hydroxy-3-(1H-imidazol-4-yl)-propionic acid, D-His, desamino-His, Nalpha-acetyl-His, or Nalpha-formyl-His
  SITE (2)..(2): This residue (Xaa8) is Ala, Ser, Aib, (1-aminocyclopropyl) carboxylic acid, or (1-aminocyclobutyl) carboxylic acid
  SITE (10)..(10): This residue (Xaa16) is Val or Leu
  SITE (12)..(12): This residue (Xaa18) is Ser or Arg
  SITE (13)..(13): This residue (Xaa19) is Tyr or Gln
  SITE (14)..(14): This residue (Xaa20) is Leu or Met
  SITE (16)..(16): This residue (Xaa22) is Gly or Glu
  SITE (17)..(17): This residue (Xaa23) is Gln, Glu, or Arg
  SITE (19)..(19): This residue (Xaa25) is Ala or Val
  SITE (20)..(20): This residue (Xaa26) is Arg or Lys
  SITE (21)..(21): This residue (Xaa27) is Glu or Leu
  SITE (24)..(24): This residue (Xaa30) is Ala or Glu
  SITE (25)..(25): This residue (Xaa31) is Trp or His
  SITE (27)..(27): This residue (Xaa33) is Val or Arg
  SITE (28)..(28): This residue (Xaa34) is Arg, Lys, His, Asn, or Gln
  SITE (29)..(29): This residue (Xaa35) is Gly or Aib
XXEGTFTSDXSXXXEXXAXXXFIXXLXXXKK

SEQ ID NO: 8 - protein, 31 aa, ARTIFICIAL
  Based on human GLP-1
  SITE (2)..(2): This amino acid residue is Aib
  SITE (30)..(30): This amino acid residue is covalently attached to a substituent
  SITE (31)..(31): This amino acid residue is covalently attached to a substituent
HXEGTFTSDVSSYLEEQAAREFIAWLVRGKK

SEQ ID NO: 9 - protein, 31 aa, ARTIFICIAL
  Based on human GLP-1
  SITE (2)..(2): This amino acid residue is Aib
  SITE (30)..(30): This amino acid residue is covalently attached to a substituent
  SITE (31)..(31): This amino acid residue is covalently attached to a substituent
HXEGTFTSDVSSYLEGQAAREFIAWLVRGKK

SEQ ID NO: 10 - protein, 31 aa, ARTIFICIAL; identical to SEQ ID NO: 8
  GLP-1 agonist based on from human GLP-1
  SITE (2)..(2): Aib
  SITE (30)..(30): This amino acid residue is covalently attached to a substituent
  SITE (31)..(31): This amino acid residue is covalently attached to a substituent